European Patent Application EP 4 470 608 A1, published December 4, 2024. Title: Lysophosphatidylserine Derivatives and Pharmaceutical Composition for Treatment or Prevention of Fibrosis comprising Lysophosphatidylserine Derivatives. Applicant: 国立大学法人東京大学. The sequence listing filed with the application follows.

SEQUENCE LISTING (22 sequences)

SEQ ID NO: 1 - DNA, 16 bp, Homo sapiens
  source 1..16: mol_type = genomic DNA
aaggtgaaggtcggag

SEQ ID NO: 2 - DNA, 16 bp, Homo sapiens
  source 1..16: mol_type = genomic DNA
aatgaaggggtcattg

SEQ ID NO: 3 - DNA, 18 bp, Homo sapiens
  source 1..18: mol_type = genomic DNA
cagccaagcactgtcagg

SEQ ID NO: 4 - DNA, 20 bp, Homo sapiens
  source 1..20: mol_type = genomic DNA
ccagagccattgtcacacac

SEQ ID NO: 5 - DNA, 20 bp, Homo sapiens
  source 1..20: mol_type = genomic DNA
aagaggaaggccaagtcgag

SEQ ID NO: 6 - DNA, 20 bp, Homo sapiens
  source 1..20: mol_type = genomic DNA
cacacgtctcggtcatggta

SEQ ID NO: 7 - DNA, 20 bp, Homo sapiens
  source 1..20: mol_type = genomic DNA
aggggagctggctacttctc

SEQ ID NO: 8 - DNA, 20 bp, Homo sapiens
  source 1..20: mol_type = genomic DNA
aggactgaccaagatgggaa

SEQ ID NO: 9 - DNA, 16 bp, Homo sapiens
  source 1..16: mol_type = genomic DNA
aaggtgaaggtcggag

SEQ ID NO: 10 - DNA, 16 bp, Homo sapiens
  source 1..16: mol_type = genomic DNA
aatgaaggggtcattg

SEQ ID NO: 11 - DNA, 18 bp, Homo sapiens
  source 1..18: mol_type = genomic DNA
cagccaagcactgtcagg

SEQ ID NO: 12 - DNA, 20 bp, Homo sapiens
  source 1..20: mol_type = genomic DNA
ccagagccattgtcacacac

SEQ ID NO: 13 - DNA, 20 bp, Homo sapiens
  source 1..20: mol_type = genomic DNA
aagaggaaggccaagtcgag

SEQ ID NO: 14 - DNA, 20 bp, Homo sapiens
  source 1..20: mol_type = genomic DNA
cacacgtctcggtcatggta

SEQ ID NO: 15 - DNA, 20 bp, Homo sapiens
  source 1..20: mol_type = genomic DNA
aggggagctggctacttctc

SEQ ID NO: 16 - DNA, 20 bp, Homo sapiens
  source 1..20: mol_type = genomic DNA
aggactgaccaagatgggaa

SEQ ID NO: 17 - DNA, 20 bp, Mus musculus
  source 1..20: mol_type = genomic DNA
tgtgtccgtcgtggatctga

SEQ ID NO: 18 - DNA, 21 bp, Mus musculus
  source 1..21: mol_type = genomic DNA
ttgctgttgaagtcgcaggag

SEQ ID NO: 19 - DNA, 21 bp, Mus musculus
  source 1..21: mol_type = genomic DNA
acatgttcagctttgtggacc

SEQ ID NO: 20 - DNA, 20 bp, Mus musculus
  source 1..20: mol_type = genomic DNA
taggccattgtgtatgcagc

SEQ ID NO: 21 - DNA, 21 bp, Mus musculus
  source 1..21: mol_type = genomic DNA
ggaacctggtttcttctcacc

SEQ ID NO: 22 - DNA, 20 bp, Mus musculus
  source 1..20: mol_type = genomic DNA
taggactgaccaaggtggct